European Patent Specification EP 4 294 385 B1, published June 17, 2026. Title: SERCA modulators and their therapeutic uses. Applicant: CNRS et al. The sequence listing filed with the application follows.

SEQUENCE LISTING (7 sequences)

SEQ ID NO: 1 - DNA, 57 bp, Artificial Sequence
  shRNAs targeting ATP2A2
ccggccaggattgaagtagcctcttctcgagaagaggctacttcaatcctggttttt

SEQ ID NO: 2 - DNA, 24 bp, Artificial Sequence
  mlFNbeta forward
ctgcgttcctgctgtgcttctcca

SEQ ID NO: 3 - DNA, 24 bp, Artificial Sequence
  mlFNbeta reverse
ttctccgtcatctccatagggatc

SEQ ID NO: 4 - DNA, 20 bp, Artificial Sequence
  mCXCL10 forward
atgacgggccagtgagaatg

SEQ ID NO: 5 - DNA, 20 bp, Artificial Sequence
  mCXCL10 reverse
tgaacacgtgggcaggatag

SEQ ID NO: 6 - DNA, 20 bp, Artificial Sequence
  mISG15 forward
gtgctccaggacggtcttac

SEQ ID NO: 7 - DNA, 20 bp, Artificial Sequence
  mISG15 reverse
ctcgctgcagttctgtacca